European Patent Specification EP 4 098 749 B1, published October 23, 2024. Title: Novel cell division membrane protein variant and a method for producing L-lysine using the same. Applicant: CJ CheilJedang Corporation. The sequence listing filed with the application follows.

SEQUENCE LISTING (10 sequences)

SEQ ID NO: 1 - protein, 441 aa, Artificial Sequence
  (I307V)_cell division membrane protein
MNTLERLKLRRTEMWLLILATLVVSIMFISLELAMGNELGTHILMLMGGYIGIFIVAHLAMAWVAPFADQIMLPVVAVLNGIGLVMIYRLDEATGYSTVNSQLMWTVVGVTLMVAVLLLLRDYKSLSRYSYLLGVVGIVLLALPLVWPQPGGVEARIWIWLGPFSIQPGEFSKILLLLFFAQLLATKRALFTVAGYRFLGMDFPRLRDLAPILVVWALAILIMAGANDFGPALLLFTTVLAMVYLATGRGSWLLIGAVLVAVGAFAVYQVSSKIQERVQNFVDPVAHYDTTGYQLSQSLFGMSWGGVTGTGIGQGYPNMIPVVHSDFILAAIGEELGLIGLAAIIVLFGVFVTRGMRTATLARDSYGKLVASGLSMTIMIQIFVVVAGISSLMPMTGLTTPFMSQGGSSLMANYILMAIILRISDSARRPVMSKQASEVAA

SEQ ID NO: 2 - DNA, 1326 bp, Artificial Sequence
  (I307V)_NCgl0043
atgaacacgcttgaacgattaaagcttcgtcgcacggaaatgtggctgctgatacttgccacactcgttgtgtcgatcatgttcatcagcctcgagctggccatgggcaatgagttgggtacccatattttgatgctgatgggcggatatatcggtatcttcatcgtcgcgcacctagccatggcatgggtggcgccgtttgctgatcaaatcatgctgcctgtggtggcggtgctcaatggcattggtttggtgatgatttatcgccttgatgaggccacgggctacagcacggtcaatagccaattgatgtggacggttgttggcgtcacgctgatggtggctgtgttgttgctgttgcgtgattacaagtcgctttcgcgttattcctacctcctcggtgtggtgggcatcgtgctgctggcgctgcctctcgtgtggccgcagccaggcggcgtggaagcccgcatctggatttggcttggacctttctccatccagccaggtgagttctccaagattttgctgctgctgttctttgctcagctgctagccaccaagcgtgctttgtttactgttgcgggctaccgtttcctcggcatggatttccctcgtttgcgtgacctcgcgccgattcttgtggtgtgggcgttggctattttgatcatggctggcgccaacgacttcggtcctgcactgctgcttttcactaccgttttggccatggtgtacctggctaccggccgtggttcctggctgttgattggtgctgtgttggtggctgtcggcgcgttcgcggtgtaccaagtttcaagcaagattcaggaacgcgtgcaaaacttcgtggatcctgtggcccactatgacaccaccggttaccagctgtcccagtccttgtttggcatgagttggggcggagtcaccggcaccggcattggtcagggttaccccaacatgatccctgtcgtgcactcggacttcattctcgcagccattggtgaggagcttggtctgattggcctggcggccatcatcgtgctgtttggtgtgtttgtcacccgcggtatgcgcaccgctaccctggctcgtgacagctacggaaagctcgtggcatctggtctgtcgatgaccatcatgatccagattttcgtcgtcgtggcaggtatttcttcactgatgcccatgacaggtttgaccactccgtttatgtcccagggtggttcatccctgatggctaactacattctgatggccatcatcttgcgtatttctgacagtgcccgccgacctgtcatgtccaagcaagcatcggaggtggctgcgtga

SEQ ID NO: 3 - protein, 441 aa, Artificial Sequence
  (WT)_cell division membrane protein
MNTLERLKLRRTEMWLLILATLVVSIMFISLELAMGNELGTHILMLMGGYIGIFIVAHLAMAWVAPFADQIMLPVVAVLNGIGLVMIYRLDEATGYSTVNSQLMWTVVGVTLMVAVLLLLRDYKSLSRYSYLLGVVGIVLLALPLVWPQPGGVEARIWIWLGPFSIQPGEFSKILLLLFFAQLLATKRALFTVAGYRFLGMDFPRLRDLAPILVVWALAILIMAGANDFGPALLLFTTVLAMVYLATGRGSWLLIGAVLVAVGAFAVYQVSSKIQERVQNFVDPVAHYDTTGYQLSQSLFGMSWGGITGTGIGQGYPNMIPVVHSDFILAAIGEELGLIGLAAIIVLFGVFVTRGMRTATLARDSYGKLVASGLSMTIMIQIFVVVAGISSLMPMTGLTTPFMSQGGSSLMANYILMAIILRISDSARRPVMSKQASEVAA

SEQ ID NO: 4 - DNA, 1326 bp, Artificial Sequence
  (WT)_NCgl0043
atgaacacgcttgaacgattaaagcttcgtcgcacggaaatgtggctgctgatacttgccacactcgttgtgtcgatcatgttcatcagcctcgagctggccatgggcaatgagttgggtacccatattttgatgctgatgggcggatatatcggtatcttcatcgtcgcgcacctagccatggcatgggtggcgccgtttgctgatcaaatcatgctgcctgtggtggcggtgctcaatggcattggtttggtgatgatttatcgccttgatgaggccacgggctacagcacggtcaatagccaattgatgtggacggttgttggcgtcacgctgatggtggctgtgttgttgctgttgcgtgattacaagtcgctttcgcgttattcctacctcctcggtgtggtgggcatcgtgctgctggcgctgcctctcgtgtggccgcagccaggcggcgtggaagcccgcatctggatttggcttggacctttctccatccagccaggtgagttctccaagattttgctgctgctgttctttgctcagctgctagccaccaagcgtgctttgtttactgttgcgggctaccgtttcctcggcatggatttccctcgtttgcgtgacctcgcgccgattcttgtggtgtgggcgttggctattttgatcatggctggcgccaacgacttcggtcctgcactgctgcttttcactaccgttttggccatggtgtacctggctaccggccgtggttcctggctgttgattggtgctgtgttggtggctgtcggcgcgttcgcggtgtaccaagtttcaagcaagattcaggaacgcgtgcaaaacttcgtggatcctgtggcccactatgacaccaccggttaccagctgtcccagtccttgtttggcatgagttggggcggaatcaccggcaccggcattggtcagggttaccccaacatgatccctgtcgtgcactcggacttcattctcgcagccattggtgaggagcttggtctgattggcctggcggccatcatcgtgctgtttggtgtgtttgtcacccgcggtatgcgcaccgctaccctggctcgtgacagctacggaaagctcgtggcatctggtctgtcgatgaccatcatgatccagattttcgtcgtcgtggcaggtatttcttcactgatgcccatgacaggtttgaccactccgtttatgtcccagggtggttcatccctgatggctaactacattctgatggccatcatcttgcgtatttctgacagtgcccgccgacctgtcatgtccaagcaagcatcggaggtggctgcgtga

SEQ ID NO: 5 - DNA, 37 bp, Artificial Sequence
  NCgl0043_1F
tgaattcgagctcggtacccggtgggcatcgtgctgc

SEQ ID NO: 6 - DNA, 33 bp, Artificial Sequence
  NCgl0043_2R
atgccggtgccggtgactccgccccaactcatg

SEQ ID NO: 7 - DNA, 33 bp, Artificial Sequence
  NCgl0043_3F
catgagttggggcggagtcaccggcaccggcat

SEQ ID NO: 8 - DNA, 37 bp, Artificial Sequence
  NCgl0043_4R
gtcgactctagaggatccccggaaaccacgtgcgttc

SEQ ID NO: 9 - DNA, 17 bp, Artificial Sequence
  NCgl0043_5F
cgggctacagcacggtc

SEQ ID NO: 10 - DNA, 17 bp, Artificial Sequence
  NCgl0043_6R
gcgagtacttggccacc